European Patent Application EP 4 201 420 A1, published June 28, 2023. Title: NON-HUMAN BACTERICIDAL/PERMEABILITY-INCREASING PROTEIN (BPI) FOR THERAPY OF INFECTIONS. Applicant: Universität Regensburg. The sequence listing filed with the application follows.

SEQUENCE LISTING (36 sequences)

SEQ ID NO: 1 - protein, 455 aa, Sebastes schlegelii
  scoBPI
INPGVKVRLTGKGLEYGRQLGMASIQQKLKTIKVPDISGKQRVSPIGKVKYSLSNMQIVDVGLPKSALDLVPGTGVKLSIGNAFLRMHGNWRVKYLRIIKDSGSFDLNVNDLTITTTIAIKSDETGRPVVSSVNCAATVGSAKIKFHGGASWLYNLFRKFVDKAIRNALQKQMCPLVANAVSDLNPQLKTLNVLAKVDQYAEIEYSMVSSPTVSNSCIDFSLKGEFYNIGKHQEPPFSPAAFSLPPQINNMLYISVSAFTINSAAFVYNTAGALSLYITDDMIPQASPIRLNTRTFGAFIPQVAKRFPGLMMKLLVKTAKNPVVTFEPNKVTVQATSTVTAYAIQPNTTLSPLFVLNLETSVSARVFVSGMRLAGAVTLNKMALTLGTSYVGEFQVRSLDSIFQVVLKVVVIPILNVQLAKGYPLPTLGKMKLVNTELQVLKDYMLIGTDVQFTG

SEQ ID NO: 2 - protein, 199 aa, Sebastes schlegelii
  N-terminus of scoBPI
INPGVKVRLTGKGLEYGRQLGMASIQQKLKTIKVPDISGKQRVSPIGKVKYSLSNMQIVDVGLPKSALDLVPGTGVKLSIGNAFLRMHGNWRVKYLRIIKDSGSFDLNVNDLTITTTIAIKSDETGRPVVSSVNCAATVGSAKIKFHGGASWLYNLFRKFVDKAIRNALQKQMCPLVANAVSDLNPQLKTLNVLAKVDQ

SEQ ID NO: 3 - protein, 97 aa, Sebastes schlegelii
  region A (partial sequence of scoBPI)
INPGVKVRLTGKGLEYGRQLGMASIQQKLKTIKVPDISGKQRVSPIGKVKYSLSNMQIVDVGLPKSALDLVPGTGVKLSIGNAFLRMHGNWRVKYLR

SEQ ID NO: 4 - protein, 38 aa, Sebastes schlegelii
  region B (partial sequence of scoBPI)
AKIKFHGGASWLYNLFRKFVDKAIRNALQKQMCPLVAN

SEQ ID NO: 5 - protein, 34 aa, Sebastes schlegelii
  region I (partial sequence of scoBPI)
GRQLGMASIQQKLKTIKVPDISGKQRVSPIGKVK

SEQ ID NO: 6 - protein, 41 aa, Sebastes schlegelii
  region II (partial sequence of scoBPI)
DVGLPKSALDLVPGTGVKLSIGNAFLRMHGNWRVKYLRIIK

SEQ ID NO: 7 - protein, 27 aa, Sebastes schlegelii
  region III (partial sequence of scoBPI)
AKIKFHGGASWLYNLFRKFVDKAIRNA

SEQ ID NO: 8 - protein, 5 aa, Sebastes schlegelii [sequence omitted]

SEQ ID NO: 9 - protein, 5 aa, Sebastes schlegelii
  sequence of interest (partial sequence of scoBPI)
QKLKT

SEQ ID NO: 10 - protein, 5 aa, Sebastes schlegelii
  sequence of interest (partial sequence of scoBPI)
GKQRV

SEQ ID NO: 11 - protein, 5 aa, Sebastes schlegelii
  sequence of interest (partial sequence of scoBPI)
GKVKY

SEQ ID NO: 12 - protein, 5 aa, Sebastes schlegelii
  sequence of interest (partial sequence of scoBPI)
LRMHG

SEQ ID NO: 13 - protein, 11 aa, Sebastes schlegelii
  sequence of interest (partial sequence of scoBPI)
WRVKYLRIIKD

SEQ ID NO: 14 - protein, 7 aa, Sebastes schlegelii
  sequence of interest (partial sequence of scoBPI)
AKIKFHG

SEQ ID NO: 15 - protein, 5 aa, Sebastes schlegelii
  sequence of interest (partial sequence of scoBPI)
KAIRN

SEQ ID NO: 16 - protein, 6 aa, Sebastes schlegelii
  sequence of interest (partial sequence of scoBPI)
IRLNTR

SEQ ID NO: 17 - protein, 7 aa, Sebastes schlegelii
  sequence of interest (partial sequence of scoBPI)
MKLLVKT

SEQ ID NO: 18 - protein, 5 aa, Sebastes schlegelii
  sequence of interest (partial sequence of scoBPI)
GKMKL

SEQ ID NO: 19 - protein, 6 aa, Artificial Sequence
  LPS binding motif
  VARIANT 1,4,6: any amino acid
  VARIANT 2,3,5: basic amino acid
XXXXXX

SEQ ID NO: 20 - protein, 7 aa, Artificial Sequence
  LPS binding motif
  VARIANT 1,4,5,7: any amino acid
  VARIANT 2,3,6: basic amino acid
XXXXXXX

SEQ ID NO: 21 - protein, 5 aa, Artificial Sequence
  glycosaminoglycan binding motif
  VARIANT 1,3,5: any amino acid
  VARIANT 2,4: basic amino acid
XXXXX

SEQ ID NO: 22 - protein, 6 aa, Artificial Sequence
  glycosaminoglycan binding motif
  VARIANT 1,3,4,6: any amino acid
  VARIANT 2,5: basic amino acid
XXXXXX

SEQ ID NO: 23 - protein, 7 aa, Artificial Sequence
  glycosaminoglycan binding motif
  VARIANT 1,3,4,5,7: any amino acid
  VARIANT 2,6: basic amino acid
XXXXXXX

SEQ ID NO: 24 - protein, 456 aa, Homo sapiens
  complete sequence (AA 1-456) of human BPI
VNPGVVVRISQKGLDYASQQGTAALQKELKRIKIPDYSDSFKIKHLGKGHYSFYSMDIREFQLPSSQISMVPNVGLKFSISNANIKISGKWKAQKRFLKMSGNFDLSIEGMSISADLKLGSNPTSGKPTITCSSCSSHINSVHVHISKSKVGWLIQLFHKKIESALRNKMNSQVCEKVTNSVSSELQPYFQTLPVMTKIDSVAGINYGLVAPPATTAETLDVQMKGEFYSENHHNPPPFAPPVMEFPAAHDRMVYLGLSDYFFNTAGLVYQEAGVLKMTLRDDMIPKESKFRLTTKFFGTFLPEVAKKFPNMKIQIHVSASTPPHLSVQPTGLTFYPAVDVQAFAVLPNSSLASLFLIGMHTTGSMEVSAESNRLVGELKLDRLLLELKHSNIGPFPVELLQDIMNYIVPILVLPRVNEKLQKGFPLPTPARVQLYNVVLQPHQNFLLFGADVVYK

SEQ ID NO: 25 - protein, 487 aa, Homo sapiens
  human BPI with signal peptide
MRENMARGPCNAPRWASLMVLVAIGTAVTAAVNPGVVVRISQKGLDYASQQGTAALQKELKRIKIPDYSDSFKIKHLGKGHYSFYSMDIREFQLPSSQISMVPNVGLKFSISNANIKISGKWKAQKRFLKMSGNFDLSIEGMSISADLKLGSNPTSGKPTITCSSCSSHINSVHVHISKSKVGWLIQLFHKKIESALRNKMNSQVCEKVTNSVSSELQPYFQTLPVMTKIDSVAGINYGLVAPPATTAETLDVQMKGEFYSENHHNPPPFAPPVMEFPAAHDRMVYLGLSDYFFNTAGLVYQEAGVLKMTLRDDMIPKESKFRLTTKFFGTFLPEVAKKFPNMKIQIHVSASTPPHLSVQPTGLTFYPAVDVQAFAVLPNSSLASLFLIGMHTTGSMEVSAESNRLVGELKLDRLLLELKHSNIGPFPVELLQDIMNYIVPILVLPRVNEKLQKGFPLPTPARVQLYNVVLQPHQNFLLFGADVVYK

SEQ ID NO: 26 - protein, 455 aa, Gadus morhua
  gaBPI
ANAGVKVKLTQKGLDFGRELAVASLQKKLMTIKVPDISGKERVKPIGKVRYSVTEMRVVKLGLPSSAIGLVPGTGFSLTITNAFLSLHGRWRVKYLRFIKDRGSFDLAIKSLSITTSISLRSDNMGLPAVAMASCTTTLGGVSVKLHGGASWLYNLFRRFIEKGLQSQLQKKLCPLVAESVSSMNQFLKTVNVMAPVDRYAEIAYPMVSSPDISSSSIGLNLKGEFYNIGNHMEPPFSPAPFFLPNQEQSMLYIGLSAFTANSASFVYNKAGTLSLKITDDMVPRSSPIRLTTNTFGVLIPQIAKLFPGLMMVLQLKMTNDPLSSIEANKVTVDAKSSLTAYAILANTKLAPLFVLNLDFSVSARVNVVGNKLAGAVTLNRLDMSLGKSYVGDFKVGSLSNIFQIVLKWVVLPTVNVRLKEGFPLPSLGKINLKNTQLQILKGYIMIGTDLQNSG

SEQ ID NO: 27 - protein, 461 aa, Acipenser baerii
  acBPI
TNPGITGRITQNGLEYGRQIGMAVLQQKLKSIKIPDMSGKEKVSPIGKVRYSLTEMQIESVSLPKSAVGLSPGTGVVLSIGNAYISIKGNWRVKYRRIVKDHGSFDLSVSGLTISAGIGVSRDETGRPTVSSASCSTSIGGVRIKFHGGASWLYNLFSKFIEKALRKALSDKICPLVSDAIGGLNPHLKTLNVLAKVDRYAEVEYSLVSPPVITKNYIDLDLKGEFYNIGQHHEPPFTAPPFSLPEQASSMLYIGVSEFTLNSAGFVYYSAGVLNTNVTDDMIAQSYPNMSVKLIVQATQQPHATMQPSNVTVEVMGSITAYVIKPDSTLAPLFILGMKASTSANLLISGKKLVGSVTLNGLVLSLQKSYVGPFQIQSLQTVLQLALKSAVLPKVNELLKEGFPLPTIDKMNLVNAQIQILKDYVLIGTDVAFTGSPARYSDTAKARYLSSVYYHYYTCLT

SEQ ID NO: 28 - protein, 455 aa, Lepisosteus oculatus
  leBPI
TNPGITVRLTQKGLEYGRQIGIAVLQQKLKSVHIPDISGKESVSPVGSVEYSLSGMQVVSLGLPQSSLVLAPGSGLSLSIGNAYISIDGNWRVKYLKFIKDHGSFDLSVSELTISAVMAVGSDETGRPTVSCTSCSASVGSAKIKFHGGASWLYNLFSSFIDKALRNALQDKLCPLVTDAIAGINPHLKTLNVLAKVDQYAEIEYSMVSSPVITKDYIDLNLKGEFYNIGKHQEPPFPAPGFSLPAQANSMLYFGVSQFTPNSAGFVYSTTGVLSINVTDDMIPKSSPLRLNTKTFGAFIPEIAKRYPGLQMELLVKSTKQPFVTFQTNNMTLQAVGSIAAYAIQPNSTLTPLFILSVDASVSGNVYVSGVKVAGSLSLNSFKLSLVTSYVGPFQVQSLSNIFQLVLKVAVLPKVNELLQQGFPLPTIEKMNLVNTQLQIQKDYLLIGTDVQFSP

SEQ ID NO: 29 - protein, 455 aa, Ictalurus punctatus
  icBPI
TNPGVILRVTQKGLEYGRQIGLVTLQKKLKTVKIPDMSGSEKVSPIGKVSYSLTGIQILDLGLPKSAVGLVPGTGVSLSIGDAYINLHGNWRVKYLRIIKDSGSFDLSVSGLSISATISVKGDDTGRPVVSSANCAASVGNVKIKFHGGASWLYNLFKHYIEKALRSELQKQICSLVAEAIEEMNPHLKTLNVLAQVDKYAEIEYSMVESPLMSNSSIDLSLKGEFYNIGQHKEPPFSPTPFSPPAQDSNMMYIGLSAFTLNSAGFVYNNAGVLSLYITDDMIPSSFPIRLNTKTFGTFIPQIAKQYPGLMMKLLVKAEKEPNVSFEPDNVTLQASSTVTAYAIQPNATLSPLFVLNVNASVSARIYVSGLTVAGNLSLDEMDMTLATSYVGPFQVKSLDSFLTMIMKAVVIPVVNALLRQGYPLPAIGNMNLVNTQLQILKDYVLIGTDVQFTG

SEQ ID NO: 30 - protein, 455 aa, Salmo trutta
  saBPI1
ANPGVKVKLTDKGIEYGKQIGMASLQQKLKTIKVPDLSGTEKVPHVGKVKYSLTGMTIVNLGLPKSALVLVPGTGVSLAITNAFINLHGNWRVRYFRFMQDRGSFDLAVNGLTITANIAIKSDETGRPMVSTVNCVANVGRASIKFHGGASWLYNLFKSYIDKALRSALQKQICPLVADAITDMNQHLKTFNVLAKVDQYAEIEYSMGTSPTISKSSMEFSLKGEFYNIVKHQEPPFSPTPFSLPPQGNNMLYIGVSSFTPNSAGFVYNNAGALSLYVTDDMIPPSSPIRLNTGTFGVFIPEIAKRFPGMMMKLLVKTVKEPTISLEPNNVTVQASGTVTAYAIQPNTTLSPLFVLNMEGSVSAQLNVTGVKLAGAITLNKIEMTLGTSYVGQFQVQSLDNIFLMVLKVVVIPKVNARLEKGFPLPSIGKMNLVNTQLQVLKDYMLIGTDVQFTG

SEQ ID NO: 31 - protein, 455 aa, Oncorhynchus mykiss
  saBPI2
ASPGVKVKLTDKGIEYGKQIGMASLQQKLKTMKVPDLSGTEKVPPIGKVKYSLTGMTIVNLGLPKSALVLMPGTGVRLAITNAFINLHGNWRVRYFRFIQDRGSFDLAVNGLTITADIAIKSDETGRPTVSTVNCVANVGSASIKFHGGASWLYNLFKSYIDKALRSALQKQICPLVADVITDMNPHLKTFNVLAKVDQYAEIEYSMVTSPTISKSSIEFSLKGEFYNIGKHQEPPFSPTPFSLPPQDNNMLYIGVSSFTPNSAGFVYNNAGALSLYVTDDMIPPSSPIRLNTGTFGVFIPEIAKRFPGMMMKLLVKTVKEPTISLEPNNVTVQASGTVTAYAIQPNTTLSPLFVLNMEGSVSAQMNVTGVKLAGAITLNKIEMTLGTSYVGQFQVQSLDNIFLMVLKVVVIPKVNARLEKGFPLPTIGKMNLINTQLQVLKDYMLIGTDVQFTG

SEQ ID NO: 32 - protein, 455 aa, Cynoglossus semilaevis
  cyBPI
TNPGVKVRLTQKGLEYGRQLGISSIQQKLRTIKVPDISGKQKVSPIGKVEYSLSNMNIVDVGLPKSAVTPVAGTGIKLSIGDAFIHLHGNWRVKYLRVIKDSGSFDLSVNALAISTSIAIHSDETGRPTVSSVSCEAHVGSVSVKFHGGASWLYNLFTNFIDKALRNTLEKQICPLVADAVSDMNPHLKTLNVIAKVDKYTEIEYSMVTSPTVSESSIDLSLKGEFYSIGKHQEAPFSPVAFFLPPQANNMLYFGISAYTPNTAAFAYNSAGALSLYITDDMIPQSSPIRLNTKTFGTFIPQIAKRYPGLMMKLLLQTIKTPNISFQPNNVTIQASATVTAYAIQPNTTLTPLFVLNLNTSVSGKMFVSEMRLAGAVTLNEMDLTLRTSYIGDFQVRSLDNILQLVLKVVVIPKLNVKLSQGYPLPAIGKMKLVNTQVQVLKDYMLVGTDVQFTG

SEQ ID NO: 33 - protein, 455 aa, Larimichthys crocea
  sciBPI
INPGVKIELTRKGLEYGRQLGMVSIQRKLKTIKIPDFSGSQSVAPIGKVQYSLSNMQIDNVQLPQSALDLVPGSGVRLSISNAFISLHGNWRVKYLKIIKDSGTFDLKVSGLSITTTIATKTDETGRPVVSTVNCSATVNSATIKFHHGASWLYNLFKKFVSKALRQAMEKKMCPLVANAVNDMNPYLKTLNVVAKVDQYAEIEYSMVSSPTIANSSVDLSLKGEFYNIGKHQEPPFSPTAFSMPPEVNNMLYIGLSAFTTNSAAFVYNKAGALSLYITDDMLPKSSPIRLNTRTFGVVIPQIAKLFPGLMMKLLVKTVKTPVITFEPSNVTVQATASVTAYAIQSNGTLTPLFVLNLDASVSAQVFVSGMRLAGAVTLNNMELTLGTSYVGEFQVKALHSIFQMVLKVVVIPKLNAQLAKGYPLPTLGKMKLVNTQLQVLKDYMLIGTDVQFKD

SEQ ID NO: 34 - protein, 455 aa, Paralichthys olivaceus
  paBPI
TNPGVKVKLTEKGLEYGRQLGMASIQQKLKTIKVPDISGKERVPPIGKVEYSLSHMQIVKLGLPKSAVDLVPGTGIKLSISNAYISLHGNWRVKYLRIIKDSGSFDLNVNGLTITSSLAIKSDETGRPTVSSVSCVATVGSVSIKFHGGASWLYNLFKNFIDKALRNALQKQICPLVADAVNELNPHLKTLNVLAKVDQYAEIEYSMVSSPTVSKSSIDLNLKGEFYNIGKHQEAPFSPTAFSLPPQNDDMLYMGMSAYSVNSAAFVYNKAGALSLYITDDMIPQSSPIRLNTRTFGTFIPEISKRFPGLMMKLLVQTVKTPVITFQPNNATTQASCTVTAYAIQPNSTLSPLFILNLETSVSAQVFISGMRVAGAVSLNKMDLTLRTSYVGEFKVRSLDNILQMVLKVVVIPKLNVQLAKGYPLPAIGKMKLVKTQLKVLKDYMLIGTDVQFTG

SEQ ID NO: 35 - protein, 456 aa, Mus musculus
  muBPI
TDPGFVAMISQKGLDFACQQGVVELQKELQAISVPDFSGVFKIKHLGKGSYEFYSMAVDGFHIPNPKIEMLPSDGLRVFIKDASIKINGKWMSRKNFLKAGGNFELSIQGVSISTDLILGSDSSGHITTICSNCDSHIDSVHIKISGSMLGWLIRLFHRKIETSLKNIIYKKICKIVRDSVSSKLQPYLKTLSVITRVDDVTSVDYSLLAPLTTTNQFLEGQLKGEFFWRGHRDPLPIHPPVMRFVPNGAYMVCMGISDYFFNTEVLAYQQSGTLKMTLGGQLLSNNGRFQLNTDFLRTFLPKVAKMFPSMGVQLLISAPVPVHLSIQPSGLSFNPKLETQAFVVLPNASLVPLFVLGMKTNASLEVDAEENRLVGEMKLGSRWLLELKESKFGPFKVEYLEDVINYLVSTLVLPKINERLRRGFPLPLPAGIRFSHFTFYPYQNFLLLEADLHLI

SEQ ID NO: 36 - protein, 458 aa, Crassostrea gigas
  osBPI
KTPGLQTRITDRALEYATEVALDILSKQVTGQQIPDQHGQSGDVKFDITGMNVKQFTKPSSRVSLIQNVGLSWSTSGTGLAIHGDFKYKYRKGIIKISDHGSFDLKASGINFQVKIEIGMDGTGRPTMKAVGCSCNVGSADIKFHGGAAWIYSLFSGQLENKLKDMVGGGNGLLCKQLNTLIDVNGMKSLQKLPVTVQIAKRFLLDYRFLSKPSFQTKFMETYHKGEVYWNAVPVDAPFAAPPLLKSSDTSRMMYIWLSDYVFNTMSYNALKYNQLQYNVTNKDLPSGVLNTTCPQSTCIGKIIKAIGTKFPNTTVMLYMKSTSMPNMTAQNGSTVVNASGDIVFFAQQPGGKYTYFLTLSATMSTTISLMIQNEKVFAKVLKLPISVTVKDSKIPVSPEGLNFIVKGIVSVFVEPKLNELGAAGFPLPVINSVHFTNTQLTVAKDTLLIATDLKYSG